European Patent Application EP 4 269 593 A1, published November 1, 2023. Title: METHOD FOR PRODUCING CHAIN UNSATURATED CARBOXYLIC ACID COMPOUND USING PHENYLALANINE AMMONIA LYASE. Applicant: RIKEN ZEON CORPORATION The Yokohama Rubber Co., Ltd. The sequence listing filed with the application follows.

SEQUENCE LISTING (16 sequences)

SEQ ID NO: 1 - DNA, 1704 bp, Anabaena variabilis
  CDS (1)..(1704)
atgaagacactatctcaagcacaaagcaaaacctcatctcaacaattttcttttactggaaattcttctgccaatgtaattattggtaatcagaaactcacaatcaatgatgttgcaagggtagcgcgtaatggcaccttagtgtctttaaccaataacactgatattttgcagggtattcaggcatcttgtgattacattaataatgctgttgaatctggggaaccaatttatggagtgacatctggttttggcggtatggccaatgttgccatatcccgtgaacaagcatctgaactccaaaccaacttagtttggttcctgaaaacaggtgcagggaacaaattacccttggcggatgtgcgcgcagctatgctcttgcgtgcaaactctcatatgcgcggtgcatctggcatcagattagaacttatcaagcgtatggagattttccttaacgctggtgtcacaccatatgtgtatgagtttggttcaattggtgcaagtggtgatttagtgccactatcctacattactggttcactgataggcttagatcccagttttaaggttgacttcaacggtaaagaaatggatgcgccaacagctctacgtcaactgaatttgtcacccttgacattgttgccgaaggaaggcttggcgatgatgaacggcacttcagtcatgacaggtattgcagcaaactgcgtctacgatactcaaattttaactgcgatcgctatgggcgttcacgctctagatatccaagctttaaacggaaccaatcaatcattccatccatttatccataattccaaaccacatcctggtcaattatgggcagcagatcagatgatttctttgttagccaattcccagttagttcgtgatgagttagatggtaaacacgattatcgtgatcacgagttgattcaagatcgttactcactccgatgccttccccagtatttggggccaatcgttgatggaatttcccagattgccaaacaaattgaaatcgaaatcaactcagtcaccgataacccactaattgatgttgataaccaagctagctatcatggaggaaatttcctcggacagtacgtgggtatgggaatggatcacctgcgttactatattgggttattggctaaacacctagatgtgcagattgccctcctcgcctcaccagagtttagcaatggactaccaccatctttattaggcaaccgagaacgtaaagtcaatatgggactcaaaggtctgcaaatatgcggtaactcaattatgccactgttgaccttctatggaaattccatcgccgatcgctttcctacccatgcagaacaatttaatcagaacatcaacagtcaaggatacacttcagcgactctagcccgccgttctgtggatatcttccagaattatgtggcgatcgctctgatgtttggagtccaagctgttgacctccgcacatataaaaagactggtcattacgatgcacgcgcctgtctatcacctgcaactgagcgcttatattcagcagtccgccacgtagttggacaaaaaccaacttcagatcgcccatatatttggaatgataatgagcaaggactggatgagcatattgcccggatttctgctgatatcgctgctggtggtgtgattgtgcaagcagttcaagatatcttaccctgcttgcattaa

SEQ ID NO: 2 - protein, 567 aa, Anabaena variabilis
MKTLSQAQSKTSSQQFSFTGNSSANVIIGNQKLTINDVARVARNGTLVSLTNNTDILQGIQASCDYINNAVESGEPIYGVTSGFGGMANVAISREQASELQTNLVWFLKTGAGNKLPLADVRAAMLLRANSHMRGASGIRLELIKRMEIFLNAGVTPYVYEFGSIGASGDLVPLSYITGSLIGLDPSFKVDFNGKEMDAPTALRQLNLSPLTLLPKEGLAMMNGTSVMTGIAANCVYDTQILTAIAMGVHALDIQALNGTNQSFHPFIHNSKPHPGQLWAADQMISLLANSQLVRDELDGKHDYRDHELIQDRYSLRCLPQYLGPIVDGISQIAKQIEIEINSVTDNPLIDVDNQASYHGGNFLGQYVGMGMDHLRYYIGLLAKHLDVQIALLASPEFSNGLPPSLLGNRERKVNMGLKGLQICGNSIMPLLTFYGNSIADRFPTHAEQFNQNINSQGYTSATLARRSVDIFQNYVAIALMFGVQAVDLRTYKKTGHYDARACLSPATERLYSAVRHVVGQKPTSDRPYIWNDNEQGLDEHIARISADIAAGGVIVQAVQDILPCLH

SEQ ID NO: 3 - DNA, 1704 bp, Artificial Sequence
  Codon-optimized AvPAL sequence
atgaaaaccctgagccaggcacagagcaaaaccagcagccagcagtttagctttaccggcaatagcagcgcaaatgtgattattggtaatcagaaactgaccatcaatgatgttgcacgtgttgcccgtaatggcaccctggttagcctgaccaataataccgatattctgcagggtattcaggccagctgtgattatatcaataatgcagttgaaagcggtgaaccgatttatggtgttaccagcggttttggtggtatggcaaatgttgcaattagccgtgaacaggcaagcgaactgcagaccaatctggtttggtttctgaaaaccggtgcaggtaataaactgccgctggcagatgttcgtgcagcaatgctgctgcgtgcaaatagccatatgcgtggtgcaagcggtattcgtctggaactgattaaacgcatggaaatctttctgaatgccggtgttaccccgtatgtttatgaatttggtagcattggtgccagcggtgatctggttccgctgagctatattaccggtagcctgattggcctggatccgagctttaaagttgattttaatggcaaagaaatggacgcaccgaccgcactgcgtcagctgaatctgagtccgctgacactgctgccgaaagaaggtctggcaatgatgaatggcaccagcgttatgaccggtattgcagcaaattgtgtttatgatacccagattctgaccgcaattgcaatgggtgttcatgcactggatattcaggcactgaatggtacaaatcagagctttcatccgtttatccataacagcaaaccgcatccgggtcagctgtgggcagcagatcagatgattagcctgctggccaatagccagctggttcgtgatgaactggatggtaaacatgattatcgtgatcatgaactgatccaggatcgttatagcctgcgttgtctgccgcagtatctgggtccgattgttgatggtattagccagattgccaagcagattgaaattgaaattaacagcgttaccgacaatccgctgattgatgttgataatcaggcaagctatcatggtggtaattttctgggtcagtatgttggtatgggtatggatcatctgcgctattatatcggtctgctggcaaaacatctggatgttcagattgcactgctggcatcaccggaatttagcaatggtctgcctccgagtctgctgggtaatcgtgaacgtaaagttaatatgggtctgaaaggtctgcagatttgcggtaatagcattatgccgctgctgaccttttatggtaatagtattgcagatcgttttccgacacatgccgaacagtttaaccagaatattaacagccagggttataccagcgcaaccctggcacgtcgtagcgttgatatttttcagaattatgttgccattgcgctgatgtttggtgttcaggcagttgatctgcgtacctacaaaaaaaccggtcattatgatgcacgtgcctgtctgtcaccggcaaccgaacgtctgtatagcgcagttcgtcatgttgttggtcagaaaccgacctcagatcgtccgtatatttggaatgataatgaacaaggcctggatgaacatattgcacgtattagtgcagatattgcagccggtggtgttattgttcaggccgttcaggacattctgccgtgtctgcattaa

SEQ ID NO: 4 - DNA, 2202 bp, Plagiochasma appendiculatum
  CDS (1)..(2202)
atggcggcgatggtgatggaagtcggtacacctgcactggaccaagtgccagcagtgaagcctctcgtcgatggggctggggactggactgtccagctgtgcctcagtccagtgccgaagtcgaatgtgaactccgaggacccattgcagtgggcaagagctgccaaaacaattcaaggcagtcactgggaggaagtgaagagcctggtgagcgagttcgagcagtcgaaggaggtggtgattcaaggagtgacactgacagttgcacaggttaccgctgtggctcgaaatcccaatgtgaccgtggtgctcgacgcagccactgccaaggagagggtggacaagagcaacgactgggtcttgcaccacatggtaaagggaactgacacttacggtgtcaccactggcttcggagccacttctcacaggcggacgaatcaaggagtggagctgcagcgagagctcatccgatttcttaatgcaggcgtgttgtctgacgatgccagcatcctacccgtgagcacgaccagagccgcgatgctggtcagaaccaacactctcatgcaggggtactccggcattcgatgggaaattttgcagaccatgcagaagcttctgaacaagcacattactcccagactccctctgcgcggaaccatcacagcctcgggggatcttgtgcccttgtcttacatcgccggactgctcaccggccgccccaactctagagcttgcacgcaggatggcaaggtgttgacctcctcggaagcactgaagcaagtaggactgctcaagccattcgagttgcagcccaaggaaggactggctatggtgaatggaaccgcggttggtgcagcgcaggcctcgatggcttgctacgatgccaacttgttggcggtgttcgcagagatttcgtccgcgctcttctgtgaagccatgcaggggaagccagaattcacagatcatttgacgcacaagctgaagcaccatccgggccagattgaagcagccgcggtgatggagtggatgctggacggaagcgcatacatgaaagcggcggccaaactgcacgagactgaccctctgaagaagcccaagcaggacaggtacgctctccgcacatcgccgcagtggttgggccctcaaattgaagtgatccgcgcggccactcactccatcgagagggagatcaactccgtgaacgacaacccgctcatcgatgtgtccagagacaaggctctgcatggaggaaatttccaaggaaccccaattggagtgtcgatggacaacatgcgcttggcgcttgctgccatagggaagctcatgttcgcacaaatgtcagaattggtgaatgatttctacaacagtggattgccgtcgaacttaacgggcggcccgaacccgagcctggactacgggttcaaaggagccgagatcgccatggcttcttactgctccgagattcagtaccttgctaatccggtgactactcacgtgcagagtgcggagcagcacaatcaggacgtgaattctctagggttgatttcggctcgcaagacggccgaagctattgaggtcctgaagctcatgtcttcaacattcatggttgcgctctgccaggctgttgatctgagacacctagaggaaaacatgctcgcaggcgtgaagcaggtggttcaacaagtcgcgaagaaaaccctctttgccgacgaggctggagtgcttcttccttctcgcttctgcgaaaaggatctgctcaaagttgtcgatgatacaccccccttcacatacgtggacgacgccaccagcaaatcgtaccctcttatgacgaaattgagggaggtgctcgtgaaccacgccatcgagaactcgaagctcgatgataagtgttcggttttccgcagaatatccgttttcgaggaggaattgaagactcagttggaagtcaccgtcccccagatcagaagccaatatgacagtggcgtcacgtccattgcgaataagatcaaggaatgccgcaccttcccgatttacaacttcgttcgatctttgggaacgaagcttctggtcggaacagagacgaggtctcctggagaggacatccagctcgtttacgaggccattaacgagggcaaatttgccagtcctttgctatcttgcttggatggttggcatggagctcccatcccaattgatgtgtga

SEQ ID NO: 5 - protein, 733 aa, Plagiochasma appendiculatum
MAAMVMEVGTPALDQVPAVKPLVDGAGDWTVQLCLSPVPKSNVNSEDPLQWARAAKTIQGSHWEEVKSLVSEFEQSKEVVIQGVTLTVAQVTAVARNPNVTVVLDAATAKERVDKSNDWVLHHMVKGTDTYGVTTGFGATSHRRTNQGVELQRELIRFLNAGVLSDDASILPVSTTRAAMLVRTNTLMQGYSGIRWEILQTMQKLLNKHITPRLPLRGTITASGDLVPLSYIAGLLTGRPNSRACTQDGKVLTSSEALKQVGLLKPFELQPKEGLAMVNGTAVGAAQASMACYDANLLAVFAEISSALFCEAMQGKPEFTDHLTHKLKHHPGQIEAAAVMEWMLDGSAYMKAAAKLHETDPLKKPKQDRYALRTSPQWLGPQIEVIRAATHSIEREINSVNDNPLIDVSRDKALHGGNFQGTPIGVSMDNMRLALAAIGKLMFAQMSELVNDFYNSGLPSNLTGGPNPSLDYGFKGAEIAMASYCSEIQYLANPVTTHVQSAEQHNQDVNSLGLISARKTAEAIEVLKLMSSTFMVALCQAVDLRHLEENMLAGVKQVVQQVAKKTLFADEAGVLLPSRFCEKDLLKVVDDTPPFTYVDDATSKSYPLMTKLREVLVNHAIENSKLDDKCSVFRRISVFEEELKTQLEVTVPQIRSQYDSGVTSIANKIKECRTFPIYNFVRSLGTKLLVGTETRSPGEDIQLVYEAINEGKFASPLLSCLDGWHGAPIPIDV

SEQ ID NO: 6 - DNA, 2203 bp, Artificial Sequence
  Codon-optimized PaPAL sequence
atggcagcaatggtaatggaagtaggtacaccagcattagatcaagtaccggcagttaaaccgctggttgatggtgccggtgattggaccgttcagctgtgtctgagtccggttccgaaaagcaatgttaatagcgaagatccgctgcagtgggcacgtgcagcaaaaaccattcagggtagccattgggaagaagttaaaagcctggttagcgaatttgaacagagcaaagaagttgttattcagggcgttaccctgaccgttgcacaggttaccgcagttgcacgtaatccgaatgttaccgttgttctggatgcagcaaccgcaaaagaacgtgttgataaaagtaatgattgggtgctgcatcatatggttaaaggcaccgatacctatggtgttaccaccggttttggtgcaaccagccatcgtcgtaccaatcagggtgttgaactgcagcgtgaactgattcgttttctgaatgccggtgttctgagtgatgatgcaagcattctgccggttagcacaacccgtgcagccatgctggttcgtacaaataccctgatgcagggttatagcggtattcgttgggaaattctgcagaccatgcagaaactgctgaacaaacatattacaccgcgtctgccgctgcgtggcaccattaccgcaagcggtgatctggttccgctgagctatattgcaggtctgctgaccggtcgtccgaatagccgtgcatgtacccaggatggtaaagttctgaccagcagcgaagcactgaaacaggttggcctgctgaaaccgtttgagctgcagccgaaagaaggtctggccatggttaatggtacagcagttggtgcagcacaggcaagcatggcatgttatgatgcaaatctgctggcagtttttgcagaaatttcaagcgcactgttttgtgaagcaatgcagggtaaaccggaatttaccgatcatctgacccataaactgaaacatcatccgggtcagattgaagcagcagcagttatggaatggatgctggatggtagcgcatatatgaaagcagccgcaaaactgcatgaaaccgatccgctgaaaaaaccgaaacaggatcgttatgcactgcgtaccagtccgcagtggctgggtccgcagatcgaagttattcgtgcagcgacccatagcattgaacgtgaaattaacagcgttaatgataacccgctgattgatgttagccgtgataaagcactgcatggtggtaattttcagggcaccccgattggtgttagcatggataatatgcgtctggcactggcagccattggtaaactgatgtttgcacagatgagcgaactggtgaatgatttctataatagcggtctgccgagtaatctgacaggcggtccgaatccgagcctggattatggttttaaaggtgccgaaattgcaatggcaagctattgtagcgaaattcagtatctggcaaatccggttaccacacatgttcagagcgcagaacagcataatcaggatgtgaatagcctgggtctgattagcgcacgtaaaaccgcagaagcaattgaagttctgaaactgatgagcagcacctttatggttgcactgtgtcaggcagttgatctgcgtcatctggaagaaaacatgctggcaggcgttaaacaggtggttcagcaggttgcaaaaaaaaccctgtttgcagatgaagcgggtgttctgctgccgagccgtttttgtgaaaaagatctgctgaaagtggttgatgatacccctccgtttacctatgttgatgatgcgaccagcaaaagctatccgctgatgaccaaactgcgtgaagtgctggttaatcatgcaatcgaaaatagcaaactggacgataaatgcagcgtgtttcgtcgtattagcgtgtttgaagaagaactgaaaacccagctggaagttaccgttccgcagattcgtagccagtatgatagcggtgtgaccagcattgccaataaaatcaaagaatgtcgcacctttccgatctataactttgttcgtagcctgggcacaaaactgctggttggtacggaaacccgtagtccgggtgaagatattcagctggtttatgaagcaatcaacgaaggtaaatttgcaagtccgctgctgagctgtctggatggttggcatggtgcaccgattccgattgatgtgtaaa

SEQ ID NO: 7 - DNA, 2124 bp, Arabidopsis thaliana
  CDS (1)..(2124)
atggagctatgcaatcaaaacaatcacatcaccgccgtctcgggcgatccgttgaactggaacgcgacggccgaagctttgaaagggagccacctggatgaggtgaaacgaatggtgaaagagtataggaaagaggcggtgaagttaggaggtgagactttgacgattggtcaagtagccgccgtggctagaggaggaggaggatctacggtggagctagcggaggaggctcgtgccggagtcaaggcgagtagcgaatgggtgatggagagcatgaaccgaggaacggacagttatggagttaccacagggtttggtgcaacttcccatagaagaaccaaacaaggcggtgcacttcaaaatgagcttattaggttcttgaatgccggaatatttggccccggcgccggggacacgtcacacacgttgccaaagccgacaacaagagcggcaatgctcgtccgtgtcaacactctcctccaaggctactccggtatacgcttcgagattctcgaagcaattacaaagcttctcaaccacgaaatcactccgtgcctccctctccgtggcaccatcaccgcctccggtgaccttgttcctctctcttacatcgccggacttctcactggccgtcccaactccaaagccgtgggtccctctggtgagactctcactgcctctgaggcctttaagctcgccggagtatcgtcctttttcgagctgcagcctaaggaaggactagcacttgtgaacgggacagcggttggatcgggtttggcctcaacggttttgttcgatgcaaatattttggctgttttatcggaagttatgtctgccatgttcgcagaggttatgcaagggaaaccggagtttacagatcatcttacgcataagctcaagcaccatcccggtcagatcgaagccgccgcaattatggaacatatattagacggaagctcttacgttaaagaagctcaacttctccacgaaatggatcctcttcaaaaacctaaacaagatcggtacgctttacgtacgtcaccacaatggcttgggccgcagattgaagtgatcagagcggctactaaaatgattgagcgtgagatcaactctgttaatgataaccctttgatagatgtgtcgaggaacaaggcgttgcacggtggaaatttccaagggacaccgatcggtgttgccatggataattcccgtctagccattgcttccattgggaaactcatgtttgcgcagttttctgaactagtgaacgatttctacaacaatggtttgccttctaatctatctggtgggagaaaccctagtcttgattacgggtttaaaggcgcggaaatagccatggcttcttattgctccgagcttcagttcctggctaatcccgtgaccaaccatgtccaaagcgcagagcagcataaccaagacgttaattccctagggctaatctctagcaggaaaactgcagaagcagtggatatcctcaagctaatgtccacaacctacttagtcgcgctttgccaagccgttgatctaagacatcttgaagagaatctgaagaaggcggttaaatcagcagtgagtcaggtggcgaaacgggtcttaaccgttggtgccaacggggagctacatccgtcaaggttcacagaacgtgatgtcctccaagtggttgaccgagagtacgtgttctcatacgcagacgatccctgcagcctcacttacccgctaatgcagaaacttagacacattcttgtagaccacgctttagcggatccagaacgcgaggccaattccgcgacatcggttttccacaaaatcggagcttttgaagccgagctgaaactgcttctccctaaagaagtagaacgcgtccgggttgaatacgaggaaggaacatcggctatagctaaccggattaaggaatgtcggtcttatccattgtatcggtttgtccgcgatgagctaaatactgaactgcttactggagagaatgttcggtcgccaggagaggagtttgataaagtgttcttagcgatttctgatggaaaacttattgatccgttgttggaatgtctcaaggagtggaacggagctccggtttcaatctgttga

SEQ ID NO: 8 - protein, 707 aa, Arabidopsis thaliana
MELCNQNNHITAVSGDPLNWNATAEALKGSHLDEVKRMVKEYRKEAVKLGGETLTIGQVAAVARGGGGSTVELAEEARAGVKASSEWVMESMNRGTDSYGVTTGFGATSHRRTKQGGALQNELIRFLNAGIFGPGAGDTSHTLPKPTTRAAMLVRVNTLLQGYSGIRFEILEAITKLLNHEITPCLPLRGTITASGDLVPLSYIAGLLTGRPNSKAVGPSGETLTASEAFKLAGVSSFFELQPKEGLALVNGTAVGSGLASTVLFDANILAVLSEVMSAMFAEVMQGKPEFTDHLTHKLKHHPGQIEAAAIMEHILDGSSYVKEAQLLHEMDPLQKPKQDRYALRTSPQWLGPQIEVIRAATKMIEREINSVNDNPLIDVSRNKALHGGNFQGTPIGVAMDNSRLAIASIGKLMFAQFSELVNDFYNNGLPSNLSGGRNPSLDYGFKGAEIAMASYCSELQFLANPVTNHVQSAEQHNQDVNSLGLISSRKTAEAVDILKLMSTTYLVALCQAVDLRHLEENLKKAVKSAVSQVAKRVLTVGANGELHPSRFTERDVLQVVDREYVFSYADDPCSLTYPLMQKLRHILVDHALADPEREANSATSVFHKIGAFEAELKLLLPKEVERVRVEYEEGTSAIANRIKECRSYPLYRFVRDELNTELLTGENVRSPGEEFDKVFLAISDGKLIDPLLECLKEWNGAPVSIC

SEQ ID NO: 9 - DNA, 2124 bp, Artificial Sequence
  Codon-optimized AtPAL sequence
atggaattatgtaatcaaaataatcatattacagcagtatcaggtgatccgctgaattggaatgcaaccgcagaagcactgaaaggtagccatctggatgaagttaaacgtatggtgaaagagtatcgtaaagaggccgttaaattaggcggtgaaaccctgaccattggccaggttgcagcagttgcacgcggtggtggtggtagcaccgttgaactggccgaagaagcacgcgcaggcgttaaagcaagcagcgaatgggttatggaaagcatgaatcgtggcaccgatagttatggtgttaccaccggttttggtgcaaccagccatcgtcgtaccaaacaaggtggtgcactgcagaatgaactgattcgttttctgaatgccggtatttttggtcctggtgccggtgataccagtcataccctgccgaaaccgaccacacgtgcagcaatgctggttcgtgttaataccctgctgcagggctatagcggtattcgttttgaaattctggaagccattaccaaactgctgaaccatgaaattaccccgtgtctgccgctgcgtggcaccattaccgcaagcggtgatctggttccgctgagctatattgcaggtctgctgaccggtcgtccgaatagcaaagcagttggtccgagtggcgaaacactgaccgccagcgaagcatttaaactggctggtgttagcagcttttttgaactgcagccgaaagaaggtctggcactggttaatggcaccgcagttggtagcggtctggcaagcaccgttctgtttgatgcaaatattctggcagttctgagcgaagttatgagcgcaatgtttgcagaagttatgcagggtaaaccggaatttaccgatcatctgacccataaactgaaacatcatccgggtcagattgaagcagcagcaattatggaacatattctggatggtagcagctatgttaaagaagcacagctgctgcacgaaatggatccgctgcagaaaccgaaacaggatcgttatgcactgcgtaccagtccgcagtggctgggtccgcagatcgaagttattcgtgccgcaaccaaaatgattgaacgtgaaattaacagcgtgaacgataacccgctgattgatgttagccgtaataaagcactgcatggtggtaattttcagggcaccccgattggtgttgcaatggataatagccgtctggccattgcaagcattggtaaactgatgtttgcacagtttagcgaactggtgaacgatttctataataacggtctgccgagcaatctgagcggtggtcgtaatccgagcctggattatggttttaaaggtgcagaaattgccatggccagctattgcagcgagctgcagtttctggcaaatccggttaccaatcatgttcagagcgcagaacagcataatcaggatgttaatagcctgggtctgattagcagccgtaaaacagcagaagccgttgatattctgaaactgatgagcaccacctatctggttgccctgtgtcaggcagttgatctgcgtcatctggaagaaaatctgaaaaaagcagttaaaagcgcagttagccaggtggcaaaacgtgttctgaccgttggtgcaaatggtgaactgcatccgtcacgttttaccgaacgtgatgttctgcaggttgttgatcgtgaatatgtttttagctatgccgatgatccgtgtagcctgacctatccgctgatgcaaaaactgcgtcatatcctggttgatcatgcactggcagatccggaacgtgaagcaaatagcgcaaccagcgtttttcataaaattggtgcatttgaagccgagctgaaactgctgctgcctaaagaagttgaacgggttcgcgttgaatatgaagaaggcaccagcgcaattgccaatcgtattaaagaatgtcgttcgtatccgctgtatcgttttgttcgtgatgaactgaatacagaactgctgacaggtgaaaatgttcgtagtccgggtgaagaatttgataaagtttttctggcgattagcgacggcaaactgattgatcctctgctggaatgtctgaaagaatggaatggtgcaccggttagcatttgctaa

SEQ ID NO: 10 - DNA, 813 bp, Artificial Sequence
  Codon-optimized PfBesC sequence
  CDS (1)..(813)
atgggtgttcgtccggttagctatctggaaaatcagcgttgtccgcgtggtagccgtaaacaggcaatgagcattacccaagaaacctttcagagcgaaaccgcatatgttgttcgtaatgaaggtgttgatctggaactgaaactgtttatggatgagcagatcgagtatatcctgaaacatcgtgcaaccgaacatccgtttctgaatgcatatgccgaacatggtctgcctccggaacagagccaggttctgtacctggaaaccctgcattatttcaaatatctgccgttttatgtgtgcggcattagcaccattacacgtgatgaagcagttctgcgtaccattgcatttaatgcccgtgatgaactgggtgaaacccatagccatagcgatctgtatcgtaaatttctgcatgataaaggcatcagcgaagaacaaatcgaagcctataaatgtctgccgagcacacaggcactgaatgatggtatttgtgcactgtatagcaaaccgcctctgcagaaagcattaggtggtctgtttgcagatgaagcaatgagcgcaagcatggttagcaaatataacgatggcctgattaaagaaggtgtgggcgaacgcggtcgttttttttggaccctgcatatggaagttgaagtgggtcatagcaatgccgtttttaacgtgatggaaaaacatctgcagacaccgcaagaacgtcgcctgtttgccgaaggtattgaacagtatctgcatctgatggaagtttattgggatggcattgaacgtaaactgaatgccggtggtcgtcagtaa

SEQ ID NO: 11 - protein, 270 aa, Artificial Sequence
  Synthetic Construct
MGVRPVSYLENQRCPRGSRKQAMSITQETFQSETAYVVRNEGVDLELKLFMDEQIEYILKHRATEHPFLNAYAEHGLPPEQSQVLYLETLHYFKYLPFYVCGISTITRDEAVLRTIAFNARDELGETHSHSDLYRKFLHDKGISEEQIEAYKCLPSTQALNDGICALYSKPPLQKALGGLFADEAMSASMVSKYNDGLIKEGVGERGRFFWTLHMEVEVGHSNAVFNVMEKHLQTPQERRLFAEGIEQYLHLMEVYWDGIERKLNAGGRQ

SEQ ID NO: 12 - DNA, 1512 bp, Saccharomyces cerevisiae
  CDS (1)..(1512): ScFDC
atgaggaagctaaatccagctttagaatttagagactttatccaggtcttaaaagatgaagatgacttaatcgaaattaccgaagagattgatccaaatctcgaagtaggtgcaattatgaggaaggcctatgaatcccacttaccagccccgttatttaaaaatctcaaaggtgcttcgaaggatcttttcagcattttaggttgcccagccggtttgagaagtaaggagaaaggagatcatggtagaattgcccatcatctggggctcgacccaaaaacaactatcaaggaaatcatagattatttgctggagtgtaaggagaaggaacctctccccccaatcactgttcctgtgtcatctgcaccttgtaaaacacatatactttctgaagaaaaaatacatctacaaagcctgccaacaccatatctacatgtttcagacggtggcaagtacttacaaacgtacggaatgtggattcttcaaactccagataaaaaatggactaattggtcaattgctagaggtatggttgtagatgacaagcatatcactggtctggtaattaaaccacaacatattagacaaattgctgactcttgggcagcaattggaaaagcaaatgaaattcctttcgcgttatgttttggcgttcccccagcagctattttagttagttccatgccaattcctgaaggtgtttctgaatcggattatgttggcgcaatcttgggtgagtcggttccagtagtaaaatgtgagaccaacgatttaatggttcctgcaacgagtgagatggtatttgagggtactttgtccttaacagatacacatctggaaggcccatttggtgagatgcatggatatgttttcaaaagccaaggtcatccttgtccattgtacactgtcaaggctatgagttacagagacaatgctattctacctgtttcgaaccccggtctttgtacggatgagacacataccttgattggttcactagtggctactgaggccaaggagctggctattgaatctggcttgccaattctggatgcctttatgccttatgaggctcaggctctttggcttatcttaaaggtggatttgaaagggctgcaagcattgaagacaacgcctgaagaattttgtaagaaggtaggtgatatttactttaggacaaaagttggttttatagtccatgaaataattttggtggcagatgatatcgacatatttaacttcaaagaagtcatctgggcctacgttacaagacatacacctgttgcagatcagatggcttttgatgatgtcacttcttttcctttggctccctttgtttcgcagtcatccagaagtaagactatgaaaggtggaaagtgcgttactaattgcatatttagacagcaatatgagcgcagttttgactacataacttgtaattttgaaaagggatatccaaaaggattagttgacaaagtaaatgaaaattggaaaaggtacggatataaataa

SEQ ID NO: 13 - protein, 503 aa, Saccharomyces cerevisiae
MRKLNPALEFRDFIQVLKDEDDLIEITEEIDPNLEVGAIMRKAYESHLPAPLFKNLKGASKDLFSILGCPAGLRSKEKGDHGRIAHHLGLDPKTTIKEIIDYLLECKEKEPLPPITVPVSSAPCKTHILSEEKIHLQSLPTPYLHVSDGGKYLQTYGMWILQTPDKKWTNWSIARGMVVDDKHITGLVIKPQHIRQIADSWAAIGKANEIPFALCFGVPPAAILVSSMPIPEGVSESDYVGAILGESVPVVKCETNDLMVPATSEMVFEGTLSLTDTHLEGPFGEMHGYVFKSQGHPCPLYTVKAMSYRDNAILPVSNPGLCTDETHTLIGSLVATEAKELAIESGLPILDAFMPYEAQALWLILKVDLKGLQALKTTPEEFCKKVGDIYFRTKVGFIVHEIILVADDIDIFNFKEVIWAYVTRHTPVADQMAFDDVTSFPLAPFVSQSSRSKTMKGGKCVTNCIFRQQYERSFDYITCNFEKGYPKGLVDKVNENWKRYGYK

SEQ ID NO: 14 - DNA, 1512 bp, Artificial Sequence
  Codon-optimized ScFDC sequence
atgcgtaaactgaatccggcactggaatttcgtgattttattcaggttctgaaagatgaggatgacctgattgaaatcaccgaagaaattgatccgaatctggaagttggtgccattatgcgtaaagcatatgaaagccatctgcctgcaccgctgtttaaaaacctgaaaggtgcaagcaaagacctgtttagcattctgggttgtccggcaggtctgcgtagcaaagaaaaaggtgatcatggtcgtattgcccatcatctgggtttagatccgaaaaccaccatcaaagagatcatcgattatctgctggaatgcaaagagaaagaaccgctgcctccgattaccgttccggttagcagcgcaccgtgtaaaacccatattctgagcgaagaaaaaatccatctgcagagcctgccgacaccgtatctgcatgtttcagatggtggtaaatatctgcagacctatggtatgtggattctgcagacaccggacaaaaaatggaccaattggagcattgcacgtggtatggttgttgatgataaacatattaccggtctggtgattaaaccgcagcatattcgtcagattgcagatagctgggcagcaattggtaaagccaatgaaattccgtttgcactgtgttttggtgttccgcctgcagcaattctggtgagcagcatgccgattccggaaggtgttagcgaaagcgattatgttggtgcgattctgggtgaaagcgttccggtggttaaatgtgaaaccaatgatctgatggttccggcaaccagcgaaatggtttttgaaggcaccctgagcctgaccgatacacatctggaaggtccgtttggtgaaatgcatggttatgtgtttaaaagccagggtcatccgtgtccgctgtataccgttaaagcaatgagctatcgtgataatgcaattctgccggtgagcaatccgggtctgtgtaccgatgaaacccatacactgattggtagcctggttgccaccgaagcaaaagaactggcaattgaaagcggtctgccgattctggatgcatttatgccgtatgaagcacaggcactgtggctgattctgaaagttgatctgaaaggactgcaggcactgaaaaccacaccggaagaattttgtaaaaaagtgggcgatatctacttccgtaccaaagttggttttatcgtgcatgaaattattctggtggccgatgatatcgacatcttcaactttaaagaagtgatttgggcatacgtgacccgtcatacaccggttgcagatcagatggcatttgatgatgttaccagctttccgctggcaccgtttgttagccagagcagccgtagcaaaacaatgaaaggtggcaaatgtgtgaccaactgtatttttcgtcagcagtatgaacgcagcttcgattatatcacctgtaactttgaaaagggctatccgaaaggtctggtggataaagttaatgaaaactggaaacgctacggctataaataa

SEQ ID NO: 15 - DNA, 570 bp, Escherichia coli
  CDS (1)..(570): Flavin prenyltransferase
atgaaacgactcattgtaggcatcagcggtgccagcggcgcgatttatggcgtgcgcttattacaggttctgcgcgatgtcacagatatcgaaacgcatctggtgatgagccaggcagcgcgccagaccttatccctcgaaacggatttttctctgcgcgaagtgcaggcattagccgatgtcacgcacgatgcgcgcgatattgccgccagcatctcttccggttctttccagacgctggggatggtgattttaccctgttcaatcaaaaccctttccggcattgtccatagctatactgatggcttactgacccgtgcggcagatgtggtgctgaaagagcgtcgcccgttggtgctctgcgtgcgtgaaacaccattgcacttaggccatctgcgtttaatgactcaggcggcagaaatcggtgcggtgattatgcctcccgttccggcgttttatcatcgcccgcaatcccttgatgatgtgataaatcagacggttaatcgtgttcttgaccagtttgcgataacccttcctgaagatctctttgcccgctggcagggcgcataa

SEQ ID NO: 16 - protein, 189 aa, Escherichia coli
MKRLIVGISGASGAIYGVRLLQVLRDVTDIETHLVMSQAARQTLSLETDFSLREVQALADVTHDARDIAASISSGSFQTLGMVILPCSIKTLSGIVHSYTDGLLTRAADVVLKERRPLVLCVRETPLHLGHLRLMTQAAEIGAVIMPPVPAFYHRPQSLDDVINQTVNRVLDQFAITLPEDLFARWQGA